European Patent Application EP 4 789 659 A1, published August 12, 2026. Title: Method of introducing molecule into lipid vesicle and cell, and dispersion formulation for antibody. Applicant: NOVIGO Pharma株式会社. The sequence listing filed with the application follows.

SEQUENCE LISTING (1 sequence)

SEQ ID NO: 1 - protein, 12 aa, synthetic construct
KKKSVYDFFVWL